European Patent Specification EP 3 704 249 B1, published May 21, 2025. Title: KITS FOR ANALYSIS USING NUCLEIC ACID ENCODING AND/OR LABEL. Applicant: Encodia, Inc. Chee, Mark S. Gunderson, Kevin Weiner, Michael Phillip Shi, Lei Muranaka, Norihito Beierle, John M. Jones, Robert C. Monfregola, Luca. Application Not Yet Assigned. The sequence listing filed with the application follows.

SEQUENCE LISTING (220 sequences)

SEQ ID NO: 1 - DNA, 15 bp, Artificial Sequence
  oligonucleotide barcode BC_1
atgtctagcatgccg

SEQ ID NO: 2 - DNA, 15 bp, Artificial Sequence
  oligonucleotide barcode BC_2
ccgtgtcatgtggaa

SEQ ID NO: 3 - DNA, 15 bp, Artificial Sequence
  oligonucleotide barcode BC_3
taagccggtatatca

SEQ ID NO: 4 - DNA, 15 bp, Artificial Sequence
  oligonucleotide barcode BC_4
ttcgatatgacggaa

SEQ ID NO: 5 - DNA, 15 bp, Artificial Sequence
  oligonucleotide barcode BC_5
cgtatacgcgttagg

SEQ ID NO: 6 - DNA, 15 bp, Artificial Sequence
  oligonucleotide barcode BC_6
aactgccgagattcc

SEQ ID NO: 7 - DNA, 15 bp, Artificial Sequence
  oligonucleotide barcode BC_7
tgatcttagctgtgc

SEQ ID NO: 8 - DNA, 15 bp, Artificial Sequence
  oligonucleotide barcode BC_8
gagtcggtaccttga

SEQ ID NO: 9 - DNA, 15 bp, Artificial Sequence
  oligonucleotide barcode BC_9
ccgcttgtgatctgg

SEQ ID NO: 10 - DNA, 15 bp, Artificial Sequence
  oligonucleotide barcode BC_10
agatagcgtaccgga

SEQ ID NO: 11 - DNA, 15 bp, Artificial Sequence
  oligonucleotide barcode BC_11
tccaggctcatcatc

SEQ ID NO: 12 - DNA, 15 bp, Artificial Sequence
  oligonucleotide barcode BC_12
gagtactagagccaa

SEQ ID NO: 13 - DNA, 15 bp, Artificial Sequence
  oligonucleotide barcode BC_13
gagcgtcaataacgg

SEQ ID NO: 14 - DNA, 15 bp, Artificial Sequence
  oligonucleotide barcode BC_14
gcggtatctacactg

SEQ ID NO: 15 - DNA, 15 bp, Artificial Sequence
  oligonucleotide barcode BC_15
cttctccgaagagaa

SEQ ID NO: 16 - DNA, 15 bp, Artificial Sequence
  oligonucleotide barcode BC_16
tgaagcctgtgttaa

SEQ ID NO: 17 - DNA, 15 bp, Artificial Sequence
  oligonucleotide barcode BC_17
ctggatggttgtcga

SEQ ID NO: 18 - DNA, 15 bp, Artificial Sequence
  oligonucleotide barcode BC_18
actgcacggttccaa

SEQ ID NO: 19 - DNA, 15 bp, Artificial Sequence
  oligonucleotide barcode BC_19
cgagagatggtcctt

SEQ ID NO: 20 - DNA, 15 bp, Artificial Sequence
  oligonucleotide barcode BC_20
tcttgagagacaaga

SEQ ID NO: 21 - DNA, 15 bp, Artificial Sequence
  oligonucleotide barcode BC_21
aattcgcactgtgtt

SEQ ID NO: 22 - DNA, 15 bp, Artificial Sequence
  oligonucleotide barcode BC_22
gtagtgccgctaaga

SEQ ID NO: 23 - DNA, 15 bp, Artificial Sequence
  oligonucleotide barcode BC_23
cctatagcacaatcc

SEQ ID NO: 24 - DNA, 15 bp, Artificial Sequence
  oligonucleotide barcode BC_24
atcaccgaggttgga

SEQ ID NO: 25 - DNA, 15 bp, Artificial Sequence
  oligonucleotide barcode BC_25
gattcaacggagaag

SEQ ID NO: 26 - DNA, 15 bp, Artificial Sequence
  oligonucleotide barcode BC_26
acgaacctcgcacca

SEQ ID NO: 27 - DNA, 15 bp, Artificial Sequence
  oligonucleotide barcode BC_27
aggacttcaagaaga

SEQ ID NO: 28 - DNA, 15 bp, Artificial Sequence
  oligonucleotide barcode BC_28
ggttgaatcctcgca

SEQ ID NO: 29 - DNA, 15 bp, Artificial Sequence
  oligonucleotide barcode BC_29
aaccaacctctagcg

SEQ ID NO: 30 - DNA, 15 bp, Artificial Sequence
  oligonucleotide barcode BC_30
acgcgaatatctaac

SEQ ID NO: 31 - DNA, 15 bp, Artificial Sequence
  oligonucleotide barcode BC_31
gttgagaattacacc

SEQ ID NO: 32 - DNA, 15 bp, Artificial Sequence
  oligonucleotide barcode BC_32
ctctctctgtgaacc

SEQ ID NO: 33 - DNA, 15 bp, Artificial Sequence
  oligonucleotide barcode BC_33
gccatcagtaagaga

SEQ ID NO: 34 - DNA, 15 bp, Artificial Sequence
  oligonucleotide barcode BC_34
gcaacgtgaattgag

SEQ ID NO: 35 - DNA, 15 bp, Artificial Sequence
  oligonucleotide barcode BC_35
ctaagtagagccaca

SEQ ID NO: 36 - DNA, 15 bp, Artificial Sequence
  oligonucleotide barcode BC_36
tgtctgttggaagcg

SEQ ID NO: 37 - DNA, 15 bp, Artificial Sequence
  oligonucleotide barcode BC_37
ttaatagacagcgcg

SEQ ID NO: 38 - DNA, 15 bp, Artificial Sequence
  oligonucleotide barcode BC_38
cgacgctctaacaag

SEQ ID NO: 39 - DNA, 15 bp, Artificial Sequence
  oligonucleotide barcode BC_39
catggcttattgaga

SEQ ID NO: 40 - DNA, 15 bp, Artificial Sequence
  oligonucleotide barcode BC_40
actaggtatggccgg

SEQ ID NO: 41 - DNA, 15 bp, Artificial Sequence
  oligonucleotide barcode BC_41
gtcctcgtctatcct

SEQ ID NO: 42 - DNA, 15 bp, Artificial Sequence
  oligonucleotide barcode BC_42
taggattccgttacc

SEQ ID NO: 43 - DNA, 15 bp, Artificial Sequence
  oligonucleotide barcode BC_43
tctgaccaccggaag

SEQ ID NO: 44 - DNA, 15 bp, Artificial Sequence
  oligonucleotide barcode BC_44
agagtcacctcgtgg

SEQ ID NO: 45 - DNA, 15 bp, Artificial Sequence
  oligonucleotide barcode BC_45
ctgatgtagtcgaag

SEQ ID NO: 46 - DNA, 15 bp, Artificial Sequence
  oligonucleotide barcode BC_46
gtcggttgcggatag

SEQ ID NO: 47 - DNA, 15 bp, Artificial Sequence
  oligonucleotide barcode BC_47
tcctcctcctaagaa

SEQ ID NO: 48 - DNA, 15 bp, Artificial Sequence
  oligonucleotide barcode BC_48
attcggtccacttca

SEQ ID NO: 49 - DNA, 15 bp, Artificial Sequence
  oligonucleotide barcode BC_49
ccttacaggtctgcg

SEQ ID NO: 50 - DNA, 15 bp, Artificial Sequence
  oligonucleotide barcode BC_50
gatcattggccaatt

SEQ ID NO: 51 - DNA, 15 bp, Artificial Sequence
  oligonucleotide barcode BC_51
ttcaaggctgagttg

SEQ ID NO: 52 - DNA, 15 bp, Artificial Sequence
  oligonucleotide barcode BC_52
tggctcgattgaatc

SEQ ID NO: 53 - DNA, 15 bp, Artificial Sequence
  oligonucleotide barcode BC_53
gtaagccatccgctc

SEQ ID NO: 54 - DNA, 15 bp, Artificial Sequence
  oligonucleotide barcode BC_54
acacatgcgtagaca

SEQ ID NO: 55 - DNA, 15 bp, Artificial Sequence
  oligonucleotide barcode BC_55
tgctatggattcaag

SEQ ID NO: 56 - DNA, 15 bp, Artificial Sequence
  oligonucleotide barcode BC_56
ccacgaggcttagtt

SEQ ID NO: 57 - DNA, 15 bp, Artificial Sequence
  oligonucleotide barcode BC_57
ggccaactaaggtgc

SEQ ID NO: 58 - DNA, 15 bp, Artificial Sequence
  oligonucleotide barcode BC_58
gcacctattcgacaa

SEQ ID NO: 59 - DNA, 15 bp, Artificial Sequence
  oligonucleotide barcode BC_59
tggacacgatcggct

SEQ ID NO: 60 - DNA, 15 bp, Artificial Sequence
  oligonucleotide barcode BC_60
ctataattccaacgg

SEQ ID NO: 61 - DNA, 15 bp, Artificial Sequence
  oligonucleotide barcode BC_61
aacgtggttagtaag

SEQ ID NO: 62 - DNA, 15 bp, Artificial Sequence
  oligonucleotide barcode BC_62
caaggaacgagtggc

SEQ ID NO: 63 - DNA, 15 bp, Artificial Sequence
  oligonucleotide barcode BC_63
caccagaacggaaga

SEQ ID NO: 64 - DNA, 15 bp, Artificial Sequence
  oligonucleotide barcode BC_64
cgtacggtcaagcaa

SEQ ID NO: 65 - DNA, 15 bp, Artificial Sequence
  oligonucleotide barcode BC_65
tcggtgacaggctaa

SEQ ID NO: 66 - DNA, 15 bp, Artificial Sequence
  oligonucleotide barcode BC_1 REV
cggcatgctagacat

SEQ ID NO: 67 - DNA, 15 bp, Artificial Sequence
  oligonucleotide barcode BC_2  REV
ttccacatgacacgg

SEQ ID NO: 68 - DNA, 15 bp, Artificial Sequence
  oligonucleotide barcode BC_3  REV
tgatataccggctta

SEQ ID NO: 69 - DNA, 15 bp, Artificial Sequence
  oligonucleotide barcode BC_4  REV
ttccgtcatatcgaa

SEQ ID NO: 70 - DNA, 15 bp, Artificial Sequence
  oligonucleotide barcode BC_5  REV
cctaacgcgtatacg

SEQ ID NO: 71 - DNA, 15 bp, Artificial Sequence
  oligonucleotide barcode BC_6  REV
ggaatctcggcagtt

SEQ ID NO: 72 - DNA, 15 bp, Artificial Sequence
  oligonucleotide barcode BC_7  REV
gcacagctaagatca

SEQ ID NO: 73 - DNA, 15 bp, Artificial Sequence
  oligonucleotide barcode BC_8  REV
tcaaggtaccgactc

SEQ ID NO: 74 - DNA, 15 bp, Artificial Sequence
  oligonucleotide barcode BC_9  REV
ccagatcacaagcgg

SEQ ID NO: 75 - DNA, 15 bp, Artificial Sequence
  oligonucleotide barcode BC_10  REV
tccggtacgctatct

SEQ ID NO: 76 - DNA, 15 bp, Artificial Sequence
  oligonucleotide barcode BC_11  REV
gatgatgagcctgga

SEQ ID NO: 77 - DNA, 15 bp, Artificial Sequence
  oligonucleotide barcode BC_12  REV
ttggctctagtactc

SEQ ID NO: 78 - DNA, 15 bp, Artificial Sequence
  oligonucleotide barcode BC_13  REV
ccgttattgacgctc

SEQ ID NO: 79 - DNA, 15 bp, Artificial Sequence
  oligonucleotide barcode BC_14  REV
cagtgtagataccgc

SEQ ID NO: 80 - DNA, 15 bp, Artificial Sequence
  oligonucleotide barcode BC_15  REV
ttctcttcggagaag

SEQ ID NO: 81 - DNA, 15 bp, Artificial Sequence
  oligonucleotide barcode BC_16  REV
ttaacacaggcttca

SEQ ID NO: 82 - DNA, 15 bp, Artificial Sequence
  oligonucleotide barcode BC_17  REV
tcgacaaccatccag

SEQ ID NO: 83 - DNA, 15 bp, Artificial Sequence
  oligonucleotide barcode BC_18  REV
ttggaaccgtgcagt

SEQ ID NO: 84 - DNA, 15 bp, Artificial Sequence
  oligonucleotide barcode BC_19 REV
aaggaccatctctcg

SEQ ID NO: 85 - DNA, 15 bp, Artificial Sequence
  oligonucleotide barcode BC_20 REV
tcttgtctctcaaga

SEQ ID NO: 86 - DNA, 15 bp, Artificial Sequence
  oligonucleotide barcode BC_21 REV
aacacagtgcgaatt

SEQ ID NO: 87 - DNA, 15 bp, Artificial Sequence
  oligonucleotide barcode BC_22 REV
tcttagcggcactac

SEQ ID NO: 88 - DNA, 15 bp, Artificial Sequence
  oligonucleotide barcode BC_23 REV
ggattgtgctatagg

SEQ ID NO: 89 - DNA, 15 bp, Artificial Sequence
  oligonucleotide barcode BC_24 REV
tccaacctcggtgat

SEQ ID NO: 90 - DNA, 15 bp, Artificial Sequence
  oligonucleotide barcode BC_25 REV
cttctccgttgaatc

SEQ ID NO: 91 - DNA, 15 bp, Artificial Sequence
  oligonucleotide barcode BC_26 REV
tggtgcgaggttcgt

SEQ ID NO: 92 - DNA, 15 bp, Artificial Sequence
  oligonucleotide barcode BC_27 REV
tcttcttgaagtcct

SEQ ID NO: 93 - DNA, 15 bp, Artificial Sequence
  oligonucleotide barcode BC_28 REV
tgcgaggattcaacc

SEQ ID NO: 94 - DNA, 15 bp, Artificial Sequence
  oligonucleotide barcode BC_29 REV
cgctagaggttggtt

SEQ ID NO: 95 - DNA, 15 bp, Artificial Sequence
  oligonucleotide barcode BC_30 REV
gttagatattcgcgt

SEQ ID NO: 96 - DNA, 15 bp, Artificial Sequence
  oligonucleotide barcode BC_31 REV
ggtgtaattctcaac

SEQ ID NO: 97 - DNA, 15 bp, Artificial Sequence
  oligonucleotide barcode BC_32 REV
ggttcacagagagag

SEQ ID NO: 98 - DNA, 15 bp, Artificial Sequence
  oligonucleotide barcode BC_33 REV
tctcttactgatggc

SEQ ID NO: 99 - DNA, 15 bp, Artificial Sequence
  oligonucleotide barcode BC_34 REV
ctcaattcacgttgc

SEQ ID NO: 100 - DNA, 15 bp, Artificial Sequence
  oligonucleotide barcode BC_35 REV
tgtggctctacttag

SEQ ID NO: 101 - DNA, 15 bp, Artificial Sequence
  oligonucleotide barcode BC_36 REV
cgcttccaacagaca

SEQ ID NO: 102 - DNA, 15 bp, Artificial Sequence
  oligonucleotide barcode BC_37 REV
cgcgctgtctattaa

SEQ ID NO: 103 - DNA, 15 bp, Artificial Sequence
  oligonucleotide barcode BC_38 REV
cttgttagagcgtcg

SEQ ID NO: 104 - DNA, 15 bp, Artificial Sequence
  oligonucleotide barcode BC_39 REV
tctcaataagccatg

SEQ ID NO: 105 - DNA, 15 bp, Artificial Sequence
  oligonucleotide barcode BC_40 REV
ccggccatacctagt

SEQ ID NO: 106 - DNA, 15 bp, Artificial Sequence
  oligonucleotide barcode BC_41 REV
aggatagacgaggac

SEQ ID NO: 107 - DNA, 15 bp, Artificial Sequence
  oligonucleotide barcode BC_42 REV
ggtaacggaatccta

SEQ ID NO: 108 - DNA, 15 bp, Artificial Sequence
  oligonucleotide barcode BC_43 REV
cttccggtggtcaga

SEQ ID NO: 109 - DNA, 15 bp, Artificial Sequence
  oligonucleotide barcode BC_44 REV
ccacgaggtgactct

SEQ ID NO: 110 - DNA, 15 bp, Artificial Sequence
  oligonucleotide barcode BC_45 REV
cttcgactacatcag

SEQ ID NO: 111 - DNA, 15 bp, Artificial Sequence
  oligonucleotide barcode BC_46 REV
ctatccgcaaccgac

SEQ ID NO: 112 - DNA, 15 bp, Artificial Sequence
  oligonucleotide barcode BC_47 REV
ttcttaggaggagga

SEQ ID NO: 113 - DNA, 15 bp, Artificial Sequence
  oligonucleotide barcode BC_48 REV
tgaagtggaccgaat

SEQ ID NO: 114 - DNA, 15 bp, Artificial Sequence
  oligonucleotide barcode BC_49 REV
cgcagacctgtaagg

SEQ ID NO: 115 - DNA, 15 bp, Artificial Sequence
  oligonucleotide barcode BC_50 REV
aattggccaatgatc

SEQ ID NO: 116 - DNA, 15 bp, Artificial Sequence
  oligonucleotide barcode BC_51 REV
caactcagccttgaa

SEQ ID NO: 117 - DNA, 15 bp, Artificial Sequence
  oligonucleotide barcode BC_52 REV
gattcaatcgagcca

SEQ ID NO: 118 - DNA, 15 bp, Artificial Sequence
  oligonucleotide barcode BC_53 REV
gagcggatggcttac

SEQ ID NO: 119 - DNA, 15 bp, Artificial Sequence
  oligonucleotide barcode BC_54 REV
tgtctacgcatgtgt

SEQ ID NO: 120 - DNA, 15 bp, Artificial Sequence
  oligonucleotide barcode BC_55 REV
cttgaatccatagca

SEQ ID NO: 121 - DNA, 15 bp, Artificial Sequence
  oligonucleotide barcode BC_56 REV
aactaagcctcgtgg

SEQ ID NO: 122 - DNA, 15 bp, Artificial Sequence
  oligonucleotide barcode BC_57 REV
gcaccttagttggcc

SEQ ID NO: 123 - DNA, 15 bp, Artificial Sequence
  oligonucleotide barcode BC_58 REV
ttgtcgaataggtgc

SEQ ID NO: 124 - DNA, 15 bp, Artificial Sequence
  oligonucleotide barcode BC_59 REV
agccgatcgtgtcca

SEQ ID NO: 125 - DNA, 15 bp, Artificial Sequence
  oligonucleotide barcode BC_60 REV
ccgttggaattatag

SEQ ID NO: 126 - DNA, 15 bp, Artificial Sequence
  oligonucleotide barcode BC_61 REV
cttactaaccacgtt

SEQ ID NO: 127 - DNA, 15 bp, Artificial Sequence
  oligonucleotide barcode BC_62 REV
gccactcgttccttg

SEQ ID NO: 128 - DNA, 15 bp, Artificial Sequence
  oligonucleotide barcode BC_63 REV
tcttccgttctggtg

SEQ ID NO: 129 - DNA, 15 bp, Artificial Sequence
  oligonucleotide barcode BC_64 REV
ttgcttgaccgtacg

SEQ ID NO: 130 - DNA, 15 bp, Artificial Sequence
  oligonucleotide barcode BC_65 REV
ttagcctgtcaccga

SEQ ID NO: 131 - protein, 16 aa, Artificial Sequence
  synthetic peptide
  MOD_RES 1: formyl-Methionine
MDVEAWLGARVPLVET

SEQ ID NO: 132 - protein, 10 aa, Artificial Sequence
  synthetic peptide
TENLYFQNHV

SEQ ID NO: 133 - DNA, 20 bp, Artificial Sequence
  oligonucleotide primer
aatgatacggcgaccaccga

SEQ ID NO: 134 - DNA, 24 bp, Artificial Sequence
  oligonucleotide primer
caagcagaagacggcatacgagat

SEQ ID NO: 135 - DNA, 5 bp, Artificial Sequence
  oligonucleotide
  misc_feature (1)...(5): n = A,T,C or G
nnnnn

SEQ ID NO: 136 - protein, 8 aa, Artificial Sequence
  synthetic peptide
DYKDDDDK

SEQ ID NO: 137 - protein, 14 aa, Artificial Sequence
  synthetic peptide
GKPIPNPLLGLDST

SEQ ID NO: 138 - protein, 10 aa, Artificial Sequence
  synthetic peptide
EQKLISEEDL

SEQ ID NO: 139 - protein, 9 aa, Artificial Sequence
  synthetic peptide
YPYDVPDYA

SEQ ID NO: 140 - protein, 9 aa, Artificial Sequence
  synthetic peptide
NWSHPQFEK

SEQ ID NO: 141 - DNA, 82 bp, Artificial Sequence
  synthetic oligonucleotide
  modified_base 1: biotin
tttttgcaaatggcattctgacatcccgtagtccgcgacactagatgtctagcatgccgccgtgtcatgtggaaactgagtg

SEQ ID NO: 142 - DNA, 72 bp, Artificial Sequence
  synthetic oligonucleotide
  modified_base 1: biotin
ttttttttttgactggttccaattgacaagccgtagtccgcgacactagtaagccggtatatcaactgagtg

SEQ ID NO: 143 - DNA, 10 bp, Artificial Sequence
  synthetic oligonucleotide
  modified_base 1: biotin
  modified_base 10: three carbon (3C) spacer
tttttttttt

SEQ ID NO: 144 - DNA, 62 bp, Artificial Sequence
  synthetic oligonucleotide
  modified_base (31)...(32): 18-atom hexa-ethyleneglycol spacer
  modified_base 62: three carbon (3C) spacer
ggatgtcagaatgccatttgcttttttttttcactcagtcctaacgcgtatacgcactcagt

SEQ ID NO: 145 - DNA, 63 bp, Artificial Sequence
  synthetic oligonucleotide
  modified_base (31)...(32): 18-atom hexa-ethyleneglycol spacer
  modified_base 63: three carbon (3C) spacer
ggatgtcagaatgccatttgcttttttttttcactcagtcctaacgcgtatacgtcactcagt

SEQ ID NO: 146 - DNA, 63 bp, Artificial Sequence; identical to SEQ ID NO: 145
  synthetic oligonucleotide
  modified_base (31)...(32): five 18-atom hexa-ethyleneglycol spacers
  modified_base 63: three carbon (3C) spacer

SEQ ID NO: 147 - DNA, 71 bp, Artificial Sequence
  synthetic oligonucleotide
  modified_base (25)...(26): 18-atom hexa-ethyleneglycol spacer
  modified_base 63: three carbon (3C) spacer)
gcttgtcaattggaaccagtcttttcactcagtcctaacgcgtatacgggaatctcggcagttcactcagt

SEQ ID NO: 148 - DNA, 44 bp, Artificial Sequence
  synthetic oligonucleotide
  modified_base 44: three carbon (3C) spacer
cgatttgcaaggatcactcgtcactcagtcctaacgcgtatacg

SEQ ID NO: 149 - DNA, 8 bp, Artificial Sequence
  spacer sequence
actgagtg

SEQ ID NO: 150 - DNA, 8 bp, Artificial Sequence
  spacer sequence
cactcagt

SEQ ID NO: 151 - DNA, 18 bp, Artificial Sequence
  oligonucleotide primer
cgtagtccgcgacactag

SEQ ID NO: 152 - DNA, 20 bp, Artificial Sequence
  oligonucleotide primer
cgatttgcaaggatcactcg

SEQ ID NO: 153 - DNA, 21 bp, Artificial Sequence
  synthetic oligonucleotide
gcaaatggcattctgacatcc

SEQ ID NO: 154 - DNA, 21 bp, Artificial Sequence
  synthetic oligonucleotide
gactggttccaattgacaagc

SEQ ID NO: 155 - DNA, 23 bp, Artificial Sequence
  synthetic oligonucleotide
  modified_base 23: three carbon (3C) spacer
cgtatacgcgttaggactgagtg

SEQ ID NO: 156 - DNA, 38 bp, Artificial Sequence
  synthetic oligonucleotide
  modified_base 38: three carbon (3C) spacer
aactgccgagattcccgtatacgcgttaggactgagtg

SEQ ID NO: 157 - DNA, 46 bp, Artificial Sequence
  oligonucleotide primer
agtccgcgcaatcagatgtctagcatgccggatccggatcgatctc

SEQ ID NO: 158 - DNA, 46 bp, Artificial Sequence
  oligonucleotide primer
agtccgcgcaatcagccgtgtcatgtggaagatccggatcgatctc

SEQ ID NO: 159 - DNA, 46 bp, Artificial Sequence
  oligonucleotide primer
agtccgcgcaatcagtaagccggtatatcagatccggatcgatctc

SEQ ID NO: 160 - DNA, 46 bp, Artificial Sequence
  oligonucleotide primer
agtccgcgcaatcagttcgatatgacggaagatccggatcgatctc

SEQ ID NO: 161 - DNA, 46 bp, Artificial Sequence
  oligonucleotide primer
tgcaaggatcactcgccagatcacaagcgggagatcgatccggatc

SEQ ID NO: 162 - DNA, 46 bp, Artificial Sequence
  oligonucleotide primer
tgcaaggatcactcgtccggtacgctatctgagatcgatccggatc

SEQ ID NO: 163 - DNA, 46 bp, Artificial Sequence
  oligonucleotide primer
tgcaaggatcactcggatgatgagcctggagagatcgatccggatc

SEQ ID NO: 164 - DNA, 46 bp, Artificial Sequence
  oligonucleotide primer
tgcaaggatcactcgttggctctagtactcgagatcgatccggatc

SEQ ID NO: 165 - DNA, 21 bp, Artificial Sequence
  oligonucleotide primer
aatcgtagtccgcgcaatcag

SEQ ID NO: 166 - DNA, 21 bp, Artificial Sequence
  oligonucleotide primer
acgatttgcaaggatcactcg

SEQ ID NO: 167 - DNA, 16 bp, Artificial Sequence
  spacer sequence
gatccggatcgatctc

SEQ ID NO: 168 - DNA, 734 bp, Artificial Sequence
  extended recording tag construct
aatcacggtacaagtcactcatccgtacgctatctgagaatcgtccagatccggcatgctagtatctggtgcagactacgattgttacagatcactcagatgatgagcacagaaaatcgtcgaatcttccatcaccatcgaacagttacgattaatgtagtccgcacaatcgaatgtctaacatgccgaatcccggacgtctccagcttctaaaccaacagtagtcgcacaaatcattgtacggtacaagatctaacgagagatgatcggatctgaccactttaaacactgattacgcagactacgattacgatttaagaatcctcgtccggtacaatcatagtccgcacaatcaaccgtgtcatgtgaagatcagatcgatctcgaatagcgtaccagacagtgatcttgcaaatcgtaatgtgtccgcgccaatcgatagccatgaatcccagtcgatctcccgcttgtgatctggcgatcgccttgtaccgtcgtacgatttgagatcacctcgttaactcaagctaaagatcgtccggatcgctttataaacatctgattgcgcggtacgattatcgtagtccgcacatatcgaacctgttgaagatccggatcgtctctccaggctcatcatccgagtgatccttgcaaataatcatgtccgcaccatcaggtgtctaacgcttgccggatccgaatcgatctctccaggctcatcatcgaagtgatgt

SEQ ID NO: 169 - protein, 10 aa, Artificial Sequence
  synthetic peptide
CPVQLWVDST

SEQ ID NO: 170 - protein, 10 aa, Artificial Sequence
  synthetic peptide
  VARIANT (1)...(10): Xaa = Any Amino Acid
CPXQXWXDXT

SEQ ID NO: 171 - protein, 8 aa, Artificial Sequence
  FLAG epitope peptide
DYKDDDDK

SEQ ID NO: 172 - protein, 14 aa, Artificial Sequence
  V5 epitope peptide
GKPIPNPLLGLDST

SEQ ID NO: 173 - protein, 10 aa, Artificial Sequence
  c-Myc epitope peptide
EQKLISEEDL

SEQ ID NO: 174 - protein, 9 aa, Artificial Sequence
  HA epitope peptide
YPYDVPDYA

SEQ ID NO: 175 - protein, 14 aa, Artificial Sequence
  V5 epitope peptide
GKPIPNPLLGLDST

SEQ ID NO: 176 - protein, 9 aa, Artificial Sequence
  StrepTag II peptide
NWSHPQFEK

SEQ ID NO: 177 - DNA, 36 bp, Artificial Sequence
  synthetic nucleotide
  misc_feature (11)...(22): compartment bar code n = A, C, T, or G
  misc_feature (23)...(27): unique molecular identifier n = A, T, C or G
gcgcaatcagnnnnnnnnnnnnnnnnntgcaaggat

SEQ ID NO: 178 - DNA, 12 bp, Artificial Sequence
  synthetic nucloetide
  misc_feature (1)...(12): Compartment barcod n = A, T, C or G
nnnnnnnnnnnn

SEQ ID NO: 179 - DNA, 5 bp, Artificial Sequence
  synthetic nucloetide
  misc_feature (1)...(5): Unique molecular identifier; n = A, T, C or G
nnnnn

SEQ ID NO: 180 - protein, 10 aa, Artificial Sequence
  butelase I peptide substrate
CGGSSGSNHV

SEQ ID NO: 181 - DNA, 47 bp, Artificial Sequence
  synthetic construct
  misc_feature 1: 5'-phosphorylated
  misc_feature 47: 3'-biotinylated
tgacatctagtgtcgcggactacgtgcttgtcaattggaaccagtct

SEQ ID NO: 182 - DNA, 49 bp, Artificial Sequence
  synthetic construct
  misc_feature 1: 5'-phosphorylated
  misc_feature 49: 3'-biotinylated
tgacatgtgaaattgttatccgctcatggatgtcagaatgccatttgct

SEQ ID NO: 183 - DNA, 49 bp, Artificial Sequence
  synthetic construct
  variation (21)...(22): 3 18-atom hexa-ethyleneglycol spacers
gactggttccaattgacaagccgatttgcaaggatcactcgutttaggt

SEQ ID NO: 184 - DNA, 76 bp, Artificial Sequence
  synthetic construct
  misc_feature 1: 5' Biotin
tttttgcaaatggcattctgacatcccgtagtccgcgacactagatgtctagcatgccgccgtgtcatgtggaaga

SEQ ID NO: 185 - DNA, 54 bp, Artificial Sequence
  synthetic construct
  misc_feature 1: 5'-phosphorylated
  misc_feature 54: 3' C3 (three carbon) spacer
ctcttcttccacatgacacggcggcatgctagacatctagtgtcgcggactacg

SEQ ID NO: 186 - DNA, 62 bp, Artificial Sequence
  synthetic construct
  variation (31)...(32): 18-atom hexa-ethyleneglycol spacer
ggatgucagaaugccatttgcttttttttttcggtctcuctcttccctaacgcgtatacgga

SEQ ID NO: 187 - DNA, 35 bp, Artificial Sequence
  synthetic construct
  misc_feature 1: 5'-phosphorylated
  misc_feature 35: 3' C3 (three carbon) spacer
agagtccgtatacgcgttagggaugagagagaccg

SEQ ID NO: 188 - DNA, 76 bp, Artificial Sequence
  synthetic construct
  variation (31)...(32): 18-atom hexa-ethyleneglycol spacer
ggatgucagaaugccatttgcttttttttttcggtctcucgatttgcaaggatcactcgccgttattgacgctcga

SEQ ID NO: 189 - DNA, 49 bp, Artificial Sequence
  synthetic construct
  misc_feature 1: 5'-phosphorylated
  misc_feature 49: 3' C3 (three carbon) spacer
agagtcgagcgtcaataacggcgagtgatccttgcaaatcgagagaccg

SEQ ID NO: 190 - DNA, 81 bp, Artificial Sequence
  synthetic construct
  misc_feature 1: 5' amine group
  variation (23)...(24): 5'-Octadiynyl dU
gcaaatggcattctgacatccttttcguaguccgcgacactagatgtctagcatgccgccgtgtcatgtggaaactgagtg

SEQ ID NO: 191 - DNA, 32 bp, Artificial Sequence
  synthetic construct
  misc_feature 1: 5' amine group 18-atom hexa-ethyleneglycol spacer
  misc_feature 32: 3' C3 (three carbon) spacer
cactcagtcctaacgcgtatacgtcactcagt

SEQ ID NO: 192 - DNA, 75 bp, Artificial Sequence
  synthetic construct
  misc_feature (31)...(32): 18-atom hexa-ethyleneglycol spacer
  misc_feature 75: 3' C3 (three carbon) spacer
ggatgtcagaatgccatttgcttttttttttcgatttgcaaggatcactcgccgttattgacgctctcactcagt

SEQ ID NO: 193 - DNA, 24 bp, Artificial Sequence
  synthetic construct
cactcagtttccacatgacacggc

SEQ ID NO: 194 - DNA, 21 bp, Artificial Sequence
  synthetic construct
cactcagtcctaacgcgtata

SEQ ID NO: 195 - protein, 18 aa, Artificial Sequence
  synthetic construct
GVAMPGAEDDVVGGGGSC

SEQ ID NO: 196 - protein, 23 aa, Artificial Sequence
  synthetic construct
  FORMYLATION 1
MDVEAWLGARVPLVETGSGSGSC

SEQ ID NO: 197 - protein, 18 aa, Artificial Sequence
  synthetic construct
HQKLVFFAEDVGSGSGSC

SEQ ID NO: 198 - protein, 103 aa, A. tumefaciens
MSDSPVDLKPKPKVKPKLERPKLYKVMLLNDDYTPREFVTVVLKAVFRMSEDTGRRVMMTAHRFGSAVVVVCERDIAETKAKEATDLGKEAGFPLMFTTEPEE

SEQ ID NO: 199 - protein, 108 aa, E. coli
MGKTNDWLDFDQLAEEKVRDALKPPSMYKVILVNDDYTPMEFVIDVLQKFFSYDVERATQLMLAVHYQGKAICGVFTAEVAETKVAMVNKYARENEHPLLCTLEKAGA

SEQ ID NO: 200 - protein, 85 aa, C. crescentus
TQKPSLYRVLILNDDYTPMEFVVYVLERFFNKSREDATRIMLHVHQNGVGVCGVYTYEVAETKVAQVIDSARRHQHPLQCTMEKD

SEQ ID NO: 201 - protein, 19 aa, Artificial Sequences
  Artificial Construct
FAGVAMPGAEDDVVGSGSK

SEQ ID NO: 202 - protein, 18 aa, Artificial Sequences
  Artificial Construct
AGVAMPGAEDDVVGSGSK

SEQ ID NO: 203 - protein, 20 aa, Artificial Sequences
  Artificial Construct
AFAGVAMPGAEDDVVGSGSK

SEQ ID NO: 204 - DNA, 22 bp, Oligonucleotide
gcttgtcaattggaaccagtct

SEQ ID NO: 205 - DNA, 23 bp, Artificial Sequences
  Oligonucleotide
gacatctagtgtcgcggactacg

SEQ ID NO: 206 - DNA, 21 bp, Artificial Sequences
  Oligonucleotide
gcttgtcaattggaaccagtc

SEQ ID NO: 207 - DNA, 24 bp, Artificial Sequences
  Oligonucleotide
cgatttgcaaggatcactcgaggt

SEQ ID NO: 208 - DNA, 22 bp, Artificial Sequences
  Oligonucleotide
gcttgtcaattggaaccagtct

SEQ ID NO: 209 - DNA, 32 bp, Artificial Sequences
  Oligonucleotide
cactcagtttccgtcatatcgaatcactcagt

SEQ ID NO: 210 - DNA, 32 bp, Artificial Sequences; identical to SEQ ID NO: 191
  Oligonucleotide

SEQ ID NO: 211 - DNA, 44 bp, Artificial Sequences
  Oligonucleotide
cgatttgcaaggatcactcgccgttattgacgctctcactcagt

SEQ ID NO: 212 - DNA, 153 bp, Artificial Sequences
  Oligonucleotide
cgtagtccgcgacactagaataagccggtatatcaactgagtgattcgatatgacggaaactgagtgacgtatacgcgttaggactgagtgagagcgtcaataacggcgagtgatccttgcaaatcgccctatagtgagtcgtattaattcgc

SEQ ID NO: 213 - DNA, 199 bp, Artificial Sequences
  Oligonucleotide
cgtagtccgcgacactagcgtatacgcgttaggactgagtgagagcgtcaataacggactgagtgagagtcggtaccttgaactgagtgaaactgccgagattccactgagtgattcgatatgacggaaactgagtgataagccggtatatcacgagtgatccttgcaaatcgccctatagtgagtcgtattaattcgc

SEQ ID NO: 214 - DNA, 70 bp, Artificial Sequences
  Oligonucleotide
gactggttccaattgacaagcttttttttcgtagtccgcgacactagtaagccggtatatcaactgagtg

SEQ ID NO: 215 - DNA, 43 bp, Artificial Sequences
  Oligonucleotide
ttcgtagtccgcgacactagtaagccggtatatcaactgagtg

SEQ ID NO: 216 - DNA, 46 bp, Artificial Sequences
  Oligonucleotide
  misc_feature (21)..(30): n is a, c, g, or t
ttcgtagtccgcgacactagnnnnnnnnnnttaagtcgactgagtg

SEQ ID NO: 217 - DNA, 46 bp, Artificial Sequences
  Oligonucleotide
  misc_feature (21)..(30): n is a, c, g, or t
ttcgtagtccgcgacactagnnnnnnnnnngttaatggactgagtg

SEQ ID NO: 218 - DNA, 46 bp, Artificial Sequences
  Oligonucleotide
  misc_feature (21)..(30): n is a, c, g, or t
ttcgtagtccgcgacactagnnnnnnnnnncagtaccgactgagtg

SEQ ID NO: 219 - DNA, 46 bp, Artificial Sequences
  Oligonucleotide
  misc_feature (21)..(30): n is a, c, g, or t
ttcgtagtccgcgacactagnnnnnnnnnngttggttaactgagtg

SEQ ID NO: 220 - DNA, 25 bp, Artificial Sequences
  Oligonucleotide
cactcagtcagactattcactcagt